European Patent Specification EP 4 196 572 B1, published July 29, 2026. Title: Immunosuppressant-resistant T-cells for adoptive immunotherapy. Applicant: Charité - Universitätsmedizin Berlin. The sequence listing filed with the application follows.

SEQUENCE LISTING (33 sequences)

SEQ ID NO: 1 - DNA, 20 bp, Homo sapiens
  Target sequence of sgRNA #2
gggcgcaccttccccaagcg

SEQ ID NO: 2 - DNA, 20 bp, Homo sapiens
  Target sequence of sgRNA #1
gcactacaccggtgagtcgg

SEQ ID NO: 3 - DNA, 20 bp, Homo sapiens
  Target sequence of sgRNA #3
cggtgagtagtggcgcgcgg

SEQ ID NO: 4 - DNA, 20 bp, Homo sapiens
  Target sequence of sgRNA #4
cgtggtataaaaggggcggg

SEQ ID NO: 5 - DNA, 20 bp, Homo sapiens
  Target sequence of sgRNA #5
cggcggtggcgtctgcaaaa

SEQ ID NO: 6 - DNA, 20 bp, Homo sapiens
  Target sequence of sgRNA #6
cgccgcccgcccgacctcaa

SEQ ID NO: 7 - DNA, 20 bp, Homo sapiens
  Target sequence of sgRNA #7
gccgcgtctcctttgaggtc

SEQ ID NO: 8 - DNA, 24 bp, Artificial Sequence
  FKBP12 amplification primer forward (sgRNA #1&2)
tctgacgggtcagataacacctag

SEQ ID NO: 9 - DNA, 20 bp, Artificial Sequence
  FKBP12 amplification primer reverse (sgRNA #1&2)
tcttccggaggcctgggttt

SEQ ID NO: 10 - DNA, 20 bp, Artificial Sequence
  FKBP12 amplification primer forward (sgRNA #3)
acagctgtatccggaggcct

SEQ ID NO: 11 - DNA, 20 bp, Artificial Sequence
  FKBP12 amplification primer reverse (sgRNA #3)
tcacagccgccgattcagac

SEQ ID NO: 12 - DNA, 21 bp, Artificial Sequence
  PPIA amplification primer (forward)
actcgcggacctcccaaaatg

SEQ ID NO: 13 - DNA, 20 bp, Artificial Sequence
  PPIA amplification primer (reverse)
acgcgcctcatcgcttgaca

SEQ ID NO: 14 - RNA, 20 nt, Artificial Sequence
  sgRNA #2 - spacer sequence of guide RNA
gggcgcaccuuccccaagcg

SEQ ID NO: 15 - RNA, 20 nt, Artificial Sequence
  sgRNA #1 - spacer sequence of guide RNA
ggacuacaccggugagucgg

SEQ ID NO: 16 - RNA, 20 nt, Artificial Sequence
  sgRNA #3 - spacer sequence of guide RNA
gggugaguaguggcgcgcgg

SEQ ID NO: 17 - RNA, 96 nt, Artificial Sequence
  sgRNA #2 - full sequence (with standard scaffold sequence for SpCas9)
gggcgcaccuuccccaagcgguuuuagagcuagaaauagcaaguuaaaauaaggcuaguccguuaucaacuugaaaaaguggcaccgagucggugc

SEQ ID NO: 18 - RNA, 96 nt, Artificial Sequence
  sgRNA #1 - full sequence (with standard scaffold sequence for SpCas9)
gcacuacaccggugagucggguuuuagagcuagaaauagcaaguuaaaauaaggcuaguccguuaucaacuugaaaaaguggcaccgagucggugc

SEQ ID NO: 19 - RNA, 96 nt, Artificial Sequence
  sgRNA #3 - full sequence (with standard scaffold sequence for SpCas9)
cggugaguaguggcgcgcggguuuuagagcuagaaauagcaaguuaaaauaaggcuaguccguuaucaacuugaaaaaguggcaccgagucggugc

SEQ ID NO: 20 - RNA, 20 nt, Artificial Sequence
  sgRNA #4 - spacer sequence of guide RNA
ggugguauaaaaggggcggg

SEQ ID NO: 21 - RNA, 20 nt, Artificial Sequence
  sgRNA #5 - spacer sequence of guide RNA
gggcgguggcgucugcaaaa

SEQ ID NO: 22 - RNA, 20 nt, Artificial Sequence
  sgRNA #6 - spacer sequence of guide RNA
ggccgcccgcccgaccucaa

SEQ ID NO: 23 - RNA, 20 nt, Artificial Sequence
  sgRNA #7 - spacer sequence of guide RNA
gccgcgucuccuuugagguc

SEQ ID NO: 24 - RNA, 96 nt, Artificial Sequence
  sgRNA #4 - full sequence (with standard scaffold sequence for SpCas9)
cgugguauaaaaggggcgggguuuuagagcuagaaauagcaaguuaaaauaaggcuaguccguuaucaacuugaaaaaguggcaccgagucggugc

SEQ ID NO: 25 - RNA, 96 nt, Artificial Sequence
  sgRNA #5 - full sequence (with standard scaffold sequence for SpCas9)
cggcgguggcgucugcaaaaguuuuagagcuagaaauagcaaguuaaaauaaggcuaguccguuaucaacuugaaaaaguggcaccgagucggugc

SEQ ID NO: 26 - RNA, 96 nt, Artificial Sequence
  sgRNA #6 - full sequence (with standard scaffold sequence for SpCas9)
cgccgcccgcccgaccucaaguuuuagagcuagaaauagcaaguuaaaauaaggcuaguccguuaucaacuugaaaaaguggcaccgagucggugc

SEQ ID NO: 27 - RNA, 96 nt, Artificial Sequence
  sgRNA #7 - full sequence (with standard scaffold sequence for SpCas9)
gccgcgucuccuuugaggucguuuuagagcuagaaauagcaaguuaaaauaaggcuaguccguuaucaacuugaaaaaguggcaccgagucggugc

SEQ ID NO: 28 - DNA, 26 bp, Artificial Sequence
  Forward primer
cgaggtactaggcagagccgtggaac

SEQ ID NO: 29 - DNA, 21 bp, Artificial Sequence
  Reverse primer
ctgtgcagcgggcataagggc

SEQ ID NO: 30 - DNA, 24 bp, Artificial Sequence
  qPCR-Forward primer
atgggagtgcaggtggaaaccatc

SEQ ID NO: 31 - DNA, 18 bp, Artificial Sequence
  qPCR-Reverse primer
cgctgggcccccgactca

SEQ ID NO: 32 - DNA, 18 bp, Artificial Sequence
  KO probe
ttccccaagcgcggccag

SEQ ID NO: 33 - DNA, 20 bp, Artificial Sequence
  control probe
agccgccgcgcgccactact